European Patent Application EP 4 786 495 A1, published August 5, 2026. Title: BDCA2单克隆抗体及其和TACI组成的融合蛋白及其方法和用途. Applicant: 南京维立志博生物科技股份有限公司. Application WO. The sequence listing filed with the application follows.

SEQUENCE LISTING (54 sequences)

SEQ ID NO: 1 - protein, 121 aa, synthetic construct
DVKLVESGGGLVKPGGSLKLSCAASGFTFSSSTMSWVRQTPEKRLEWVATTGGGGSYTYNPDSVKGRFTISRDNAKNTLYLQMSSLRSEDTAMYYCTRDRYDGYYFSMDFWGQGTSVTVSS

SEQ ID NO: 2 - protein, 111 aa, synthetic construct
DIVLTQSPASLAVSLGQRATISCKASQSVDYDGDSYMNWYQQKPGQPPKLLIYAASNLESGIPARFSGSGSGTDFTLNIHPVEEEDAATYYCQQSNEDPRTFGGGTKLEIK

SEQ ID NO: 3 - protein, 121 aa, synthetic construct
QVLLQQSGPELVRPGVSVKVSCKGSGYTFTDFAVHWVKQSQTKSLEWIGLIGTSSGSTNYNQKFKDKATMTVDKSSNTAYLELARLTSEDSAIYYCARNGYYVGYYALDYWGQGTSVTVSS

SEQ ID NO: 4 - protein, 106 aa, synthetic construct
QTVLTQSPAIMSASPGEKVTITCSASSSVSYMYWFQQKPGTSPKLWIYSTSNLASGVPPRFSGSGSGTSYSLTISRMEAEDAATYYCQQRRNYPHTFGGGTKLEIK

SEQ ID NO: 5 - protein, 330 aa, synthetic construct [sequence omitted]

SEQ ID NO: 6 - protein, 107 aa, synthetic construct [sequence omitted]

SEQ ID NO: 7 - protein, 452 aa, synthetic construct
DVQLVESGGGLVKPGGSLRLSCAASGFTFSTYTMSWVRQAPGKGLEWVATISPGDSFGYYYPDSVQGRFTISRDNAKNSLYLQMNSLRAEDTAVYYCTRDIYYNYGAWFAYWGQGTLVTVSSASTKGPSVFPLAPSSKSTSGGTAALGCLVKDYFPEPVTVSWNSGALTSGVHTFPAVLQSSGLYSLSSVVTVPSSSLGTQTYICNVNHKPSNTKVDKKVEPKSCDKTHTCPPCPAPELLGGPSVFLFPPKPKDTLMISRTPEVTCVVVDVSHEDPEVKFNWYVDGVEVHNAKTKPREEQYNSTYRVVSVLTVLHQDWLNGKEYKCKVSNKALPAPIEKTISKAKGQPREPQVYTLPPSRDELTKNQVSLTCLVKGFYPSDIAVEWESNGQPENNYKTTPPVLDSDGSFFLYSKLTVDKSRWQQGNVFSCSVMHEALHNHYTQKSLSLSPGK

SEQ ID NO: 8 - protein, 218 aa, synthetic construct
DIQLTQSPSSLSASVGDRVTITCKASQSVDYDGDSYMNWYQQKPGKAPKLLIYAASTLESGVPSRFSGSGSGTDFTLTISSLQPEDFATYYCQQANEDPRTFGQGTKVEIKRTVAAPSVFIFPPSDEQLKSGTASVVCLLNNFYPREAKVQWKVDNALQSGNSQESVTEQDSKDSTYSLSSTLTLSKADYEKHKVYACEVTHQGLSSPVTKSFNRGEC

SEQ ID NO: 9 - protein, 451 aa, synthetic construct
DVKLVESGGGLVKPGGSLKLSCAASGFTFSSSTMSWVRQTPEKRLEWVATTGGGGSYTYNPDSVKGRFTISRDNAKNTLYLQMSSLRSEDTAMYYCTRDRYDGYYFSMDFWGQGTSVTVSSASTKGPSVFPLAPSSKSTSGGTAALGCLVKDYFPEPVTVSWNSGALTSGVHTFPAVLQSSGLYSLSSVVTVPSSSLGTQTYICNVNHKPSNTKVDKKVEPKSCDKTHTCPPCPAPELLGGPSVFLFPPKPKDTLMISRTPEVTCVVVDVSHEDPEVKFNWYVDGVEVHNAKTKPREEQYNSTYRVVSVLTVLHQDWLNGKEYKCKVSNKALPAPIEKTISKAKGQPREPQVYTLPPSRDELTKNQVSLTCLVKGFYPSDIAVEWESNGQPENNYKTTPPVLDSDGSFFLYSKLTVDKSRWQQGNVFSCSVMHEALHNHYTQKSLSLSPGK

SEQ ID NO: 10 - protein, 218 aa, synthetic construct
DIVLTQSPASLAVSLGQRATISCKASQSVDYDGDSYMNWYQQKPGQPPKLLIYAASNLESGIPARFSGSGSGTDFTLNIHPVEEEDAATYYCQQSNEDPRTFGGGTKLEIKRTVAAPSVFIFPPSDEQLKSGTASVVCLLNNFYPREAKVQWKVDNALQSGNSQESVTEQDSKDSTYSLSSTLTLSKADYEKHKVYACEVTHQGLSSPVTKSFNRGEC

SEQ ID NO: 11 - protein, 451 aa, synthetic construct
QVLLQQSGPELVRPGVSVKVSCKGSGYTFTDFAVHWVKQSQTKSLEWIGLIGTSSGSTNYNQKFKDKATMTVDKSSNTAYLELARLTSEDSAIYYCARNGYYVGYYALDYWGQGTSVTVSSASTKGPSVFPLAPSSKSTSGGTAALGCLVKDYFPEPVTVSWNSGALTSGVHTFPAVLQSSGLYSLSSVVTVPSSSLGTQTYICNVNHKPSNTKVDKKVEPKSCDKTHTCPPCPAPELLGGPSVFLFPPKPKDTLMISRTPEVTCVVVDVSHEDPEVKFNWYVDGVEVHNAKTKPREEQYNSTYRVVSVLTVLHQDWLNGKEYKCKVSNKALPAPIEKTISKAKGQPREPQVYTLPPSRDELTKNQVSLTCLVKGFYPSDIAVEWESNGQPENNYKTTPPVLDSDGSFFLYSKLTVDKSRWQQGNVFSCSVMHEALHNHYTQKSLSLSPGK

SEQ ID NO: 12 - protein, 213 aa, synthetic construct
QTVLTQSPAIMSASPGEKVTITCSASSSVSYMYWFQQKPGTSPKLWIYSTSNLASGVPPRFSGSGSGTSYSLTISRMEAEDAATYYCQQRRNYPHTFGGGTKLEIKRTVAAPSVFIFPPSDEQLKSGTASVVCLLNNFYPREAKVQWKVDNALQSGNSQESVTEQDSKDSTYSLSSTLTLSKADYEKHKVYACEVTHQGLSSPVTKSFNRGEC

SEQ ID NO: 13 - protein, 121 aa, synthetic construct
QVQLVQSGAEVKKPGASVKVSCKASGYTFTDFAVHWVRQAPGQRLEWMGLIGTSSGSTNYNQKFQGRVTMTVDKSANTAYMELSSLRSEDTAVYYCARNGYYVGYYALDYWGQGTTVTVSS

SEQ ID NO: 14 - protein, 121 aa, synthetic construct
QVQLVQSGAEVKKPGASVKVSCKASGYTFTDFAVHWVRQAPGQRLEWMGLIGTSSGSTNYNQKFQGRATMTVDKSANTAYMELSSLRSEDTAVYYCARNGYYVGYYALDYWGQGTTVTVSS

SEQ ID NO: 15 - protein, 106 aa, synthetic construct
ETVLTQSPATLSLSPGERATLSCRASSSVSYMYWFQQKPGQAPRLLIYSTSNLASGIPARFSGSGSGTDYTLTISSLEPEDFAVYYCQQRRNYPHTFGGGTKVEIK

SEQ ID NO: 16 - protein, 451 aa, synthetic construct
QVQLVQSGAEVKKPGASVKVSCKASGYTFTDFAVHWVRQAPGQRLEWMGLIGTSSGSTNYNQKFQGRVTMTVDKSANTAYMELSSLRSEDTAVYYCARNGYYVGYYALDYWGQGTTVTVSSASTKGPSVFPLAPSSKSTSGGTAALGCLVKDYFPEPVTVSWNSGALTSGVHTFPAVLQSSGLYSLSSVVTVPSSSLGTQTYICNVNHKPSNTKVDKKVEPKSCDKTHTCPPCPAPELLGGPSVFLFPPKPKDTLMISRTPEVTCVVVDVSHEDPEVKFNWYVDGVEVHNAKTKPREEQYNSTYRVVSVLTVLHQDWLNGKEYKCKVSNKALPAPIEKTISKAKGQPREPQVYTLPPSRDELTKNQVSLTCLVKGFYPSDIAVEWESNGQPENNYKTTPPVLDSDGSFFLYSKLTVDKSRWQQGNVFSCSVMHEALHNHYTQKSLSLSPGK

SEQ ID NO: 17 - protein, 451 aa, synthetic construct
QVQLVQSGAEVKKPGASVKVSCKASGYTFTDFAVHWVRQAPGQRLEWMGLIGTSSGSTNYNQKFQGRATMTVDKSANTAYMELSSLRSEDTAVYYCARNGYYVGYYALDYWGQGTTVTVSSASTKGPSVFPLAPSSKSTSGGTAALGCLVKDYFPEPVTVSWNSGALTSGVHTFPAVLQSSGLYSLSSVVTVPSSSLGTQTYICNVNHKPSNTKVDKKVEPKSCDKTHTCPPCPAPELLGGPSVFLFPPKPKDTLMISRTPEVTCVVVDVSHEDPEVKFNWYVDGVEVHNAKTKPREEQYNSTYRVVSVLTVLHQDWLNGKEYKCKVSNKALPAPIEKTISKAKGQPREPQVYTLPPSRDELTKNQVSLTCLVKGFYPSDIAVEWESNGQPENNYKTTPPVLDSDGSFFLYSKLTVDKSRWQQGNVFSCSVMHEALHNHYTQKSLSLSPGK

SEQ ID NO: 18 - protein, 213 aa, synthetic construct
ETVLTQSPATLSLSPGERATLSCRASSSVSYMYWFQQKPGQAPRLLIYSTSNLASGIPARFSGSGSGTDYTLTISSLEPEDFAVYYCQQRRNYPHTFGGGTKVEIKRTVAAPSVFIFPPSDEQLKSGTASVVCLLNNFYPREAKVQWKVDNALQSGNSQESVTEQDSKDSTYSLSSTLTLSKADYEKHKVYACEVTHQGLSSPVTKSFNRGEC

SEQ ID NO: 19 - protein, 333 aa, synthetic construct
SRVDQEERFPQGLWTGVAMRSCPEEQYWDPLLGTCMSCKTICNHQSQRTCAAFCRSLSCRKEQGKFYDHLLRDCISCASICGQHPKQCAYFCENKLRSPVNLPPELDKTHTCPPCPAPEAEGAPSVFLFPPKPKDTLMISRTPEVTCVVVDVSHEDPEVKFNWYVDGVEVHNAKTKPREEQYNSTYRVVSVLTVLHQDWLNGKEYKCKVSNKALPSSIEKTISKAKGQPREPQVYTLPPSRDELTKNQVSLTCLVKGFYPSDIAVEWESNGQPENNYKTTPPVLDSDGSFFLYSKLTVDKSRWQQGNVFSCSVMHEALHNHYTQKSLSLSPGK

SEQ ID NO: 20 - protein, 106 aa, synthetic construct
SRVDQEERFPQGLWTGVAMRSCPEEQYWDPLLGTCMSCKTICNHQSQRTCAAFCRSLSCRKEQGKFYDHLLRDCISCASICGQHPKQCAYFCENKLRSPVNLPPEL

SEQ ID NO: 21 - protein, 39 aa, synthetic construct
SLSCRKEQGKFYDHLLRDCISCASICGQHPKQCAYFCEN

SEQ ID NO: 22 - protein, 505 aa, synthetic construct
QVQLVQSGAEVKKPGASVKVSCKASGYTFTDFAVHWVRQAPGQRLEWMGLIGTSSGSTNYNQKFQGRATMTVDKSANTAYMELSSLRSEDTAVYYCARNGYYVGYYALDYWGQGTTVTVSSASTKGPSVFPLAPSSKSTSGGTAALGCLVKDYFPEPVTVSWNSGALTSGVHTFPAVLQSSGLYSLSSVVTVPSSSLGTQTYICNVNHKPSNTKVDKKVEPKSCDKTHTCPPCPAPELLGGPSVFLFPPKPKDTLMISRTPEVTCVVVDVSHEDPEVKFNWYVDGVEVHNAKTKPREEQYNSTYRVVSVLTVLHQDWLNGKEYKCKVSNKALPAPIEKTISKAKGQPREPQVYTLPPSRDELTKNQVSLTCLVKGFYPSDIAVEWESNGQPENNYKTTPPVLDSDGSFFLYSKLTVDKSRWQQGNVFSCSVMHEALHNHYTQKSLSLSPGKGGGGSGGGGSGGGGSSLSCRKEQGKFYDHLLRDCISCASICGQHPKQCAYFCEN

SEQ ID NO: 23 - protein, 505 aa, synthetic construct
SLSCRKEQGKFYDHLLRDCISCASICGQHPKQCAYFCENGGGGSGGGGSGGGGSQVQLVQSGAEVKKPGASVKVSCKASGYTFTDFAVHWVRQAPGQRLEWMGLIGTSSGSTNYNQKFQGRATMTVDKSANTAYMELSSLRSEDTAVYYCARNGYYVGYYALDYWGQGTTVTVSSASTKGPSVFPLAPSSKSTSGGTAALGCLVKDYFPEPVTVSWNSGALTSGVHTFPAVLQSSGLYSLSSVVTVPSSSLGTQTYICNVNHKPSNTKVDKKVEPKSCDKTHTCPPCPAPELLGGPSVFLFPPKPKDTLMISRTPEVTCVVVDVSHEDPEVKFNWYVDGVEVHNAKTKPREEQYNSTYRVVSVLTVLHQDWLNGKEYKCKVSNKALPAPIEKTISKAKGQPREPQVYTLPPSRDELTKNQVSLTCLVKGFYPSDIAVEWESNGQPENNYKTTPPVLDSDGSFFLYSKLTVDKSRWQQGNVFSCSVMHEALHNHYTQKSLSLSPGK

SEQ ID NO: 24 - protein, 572 aa, synthetic construct
SRVDQEERFPQGLWTGVAMRSCPEEQYWDPLLGTCMSCKTICNHQSQRTCAAFCRSLSCRKEQGKFYDHLLRDCISCASICGQHPKQCAYFCENKLRSPVNLPPELGGGGSGGGGSGGGGSQVQLVQSGAEVKKPGASVKVSCKASGYTFTDFAVHWVRQAPGQRLEWMGLIGTSSGSTNYNQKFQGRATMTVDKSANTAYMELSSLRSEDTAVYYCARNGYYVGYYALDYWGQGTTVTVSSASTKGPSVFPLAPSSKSTSGGTAALGCLVKDYFPEPVTVSWNSGALTSGVHTFPAVLQSSGLYSLSSVVTVPSSSLGTQTYICNVNHKPSNTKVDKKVEPKSCDKTHTCPPCPAPELLGGPSVFLFPPKPKDTLMISRTPEVTCVVVDVSHEDPEVKFNWYVDGVEVHNAKTKPREEQYNSTYRVVSVLTVLHQDWLNGKEYKCKVSNKALPAPIEKTISKAKGQPREPQVYTLPPSRDELTKNQVSLTCLVKGFYPSDIAVEWESNGQPENNYKTTPPVLDSDGSFFLYSKLTVDKSRWQQGNVFSCSVMHEALHNHYTQKSLSLSPGK

SEQ ID NO: 25 - protein, 500 aa, synthetic construct
SLSCRKEQGKFYDHLLRDCISCASICGQHPKQCAYFCENGSSSSGSSSSQVQLVQSGAEVKKPGASVKVSCKASGYTFTDFAVHWVRQAPGQRLEWMGLIGTSSGSTNYNQKFQGRATMTVDKSANTAYMELSSLRSEDTAVYYCARNGYYVGYYALDYWGQGTTVTVSSASTKGPSVFPLAPSSKSTSGGTAALGCLVKDYFPEPVTVSWNSGALTSGVHTFPAVLQSSGLYSLSSVVTVPSSSLGTQTYICNVNHKPSNTKVDKKVEPKSCDKTHTCPPCPAPELLGGPSVFLFPPKPKDTLMISRTPEVTCVVVDVSHEDPEVKFNWYVDGVEVHNAKTKPREEQYNSTYRVVSVLTVLHQDWLNGKEYKCKVSNKALPAPIEKTISKAKGQPREPQVYTLPPSRDELTKNQVSLTCLVKGFYPSDIAVEWESNGQPENNYKTTPPVLDSDGSFFLYSKLTVDKSRWQQGNVFSCSVMHEALHNHYTQKSLSLSPGK

SEQ ID NO: 26 - protein, 505 aa, synthetic construct
SLSCRKEQGKFYDHLLRDCISCASICGQHPKQCAYFCENGSSSSGSSSSGSSSSQVQLVQSGAEVKKPGASVKVSCKASGYTFTDFAVHWVRQAPGQRLEWMGLIGTSSGSTNYNQKFQGRATMTVDKSANTAYMELSSLRSEDTAVYYCARNGYYVGYYALDYWGQGTTVTVSSASTKGPSVFPLAPSSKSTSGGTAALGCLVKDYFPEPVTVSWNSGALTSGVHTFPAVLQSSGLYSLSSVVTVPSSSLGTQTYICNVNHKPSNTKVDKKVEPKSCDKTHTCPPCPAPELLGGPSVFLFPPKPKDTLMISRTPEVTCVVVDVSHEDPEVKFNWYVDGVEVHNAKTKPREEQYNSTYRVVSVLTVLHQDWLNGKEYKCKVSNKALPAPIEKTISKAKGQPREPQVYTLPPSRDELTKNQVSLTCLVKGFYPSDIAVEWESNGQPENNYKTTPPVLDSDGSFFLYSKLTVDKSRWQQGNVFSCSVMHEALHNHYTQKSLSLSPGK

SEQ ID NO: 27 - protein, 510 aa, synthetic construct
SLSCRKEQGKFYDHLLRDCISCASICGQHPKQCAYFCENGSSSSGSSSSGSSSSGSSSSQVQLVQSGAEVKKPGASVKVSCKASGYTFTDFAVHWVRQAPGQRLEWMGLIGTSSGSTNYNQKFQGRATMTVDKSANTAYMELSSLRSEDTAVYYCARNGYYVGYYALDYWGQGTTVTVSSASTKGPSVFPLAPSSKSTSGGTAALGCLVKDYFPEPVTVSWNSGALTSGVHTFPAVLQSSGLYSLSSVVTVPSSSLGTQTYICNVNHKPSNTKVDKKVEPKSCDKTHTCPPCPAPELLGGPSVFLFPPKPKDTLMISRTPEVTCVVVDVSHEDPEVKFNWYVDGVEVHNAKTKPREEQYNSTYRVVSVLTVLHQDWLNGKEYKCKVSNKALPAPIEKTISKAKGQPREPQVYTLPPSRDELTKNQVSLTCLVKGFYPSDIAVEWESNGQPENNYKTTPPVLDSDGSFFLYSKLTVDKSRWQQGNVFSCSVMHEALHNHYTQKSLSLSPGK

SEQ ID NO: 28 - protein, 495 aa, synthetic construct
QVQLVQSGAEVKKPGASVKVSCKASGYTFTDFAVHWVRQAPGQRLEWMGLIGTSSGSTNYNQKFQGRATMTVDKSANTAYMELSSLRSEDTAVYYCARNGYYVGYYALDYWGQGTTVTVSSASTKGPSVFPLAPSSKSTSGGTAALGCLVKDYFPEPVTVSWNSGALTSGVHTFPAVLQSSGLYSLSSVVTVPSSSLGTQTYICNVNHKPSNTKVDKKVEPKSCDKTHTCPPCPAPELLGGPSVFLFPPKPKDTLMISRTPEVTCVVVDVSHEDPEVKFNWYVDGVEVHNAKTKPREEQYNSTYRVVSVLTVLHQDWLNGKEYKCKVSNKALPAPIEKTISKAKGQPREPQVYTLPPSRDELTKNQVSLTCLVKGFYPSDIAVEWESNGQPENNYKTTPPVLDSDGSFFLYSKLTVDKSRWQQGNVFSCSVMHEALHNHYTQKSLSLSPGKGSSSSSLSCRKEQGKFYDHLLRDCISCASICGQHPKQCAYFCEN

SEQ ID NO: 29 - protein, 500 aa, synthetic construct
QVQLVQSGAEVKKPGASVKVSCKASGYTFTDFAVHWVRQAPGQRLEWMGLIGTSSGSTNYNQKFQGRATMTVDKSANTAYMELSSLRSEDTAVYYCARNGYYVGYYALDYWGQGTTVTVSSASTKGPSVFPLAPSSKSTSGGTAALGCLVKDYFPEPVTVSWNSGALTSGVHTFPAVLQSSGLYSLSSVVTVPSSSLGTQTYICNVNHKPSNTKVDKKVEPKSCDKTHTCPPCPAPELLGGPSVFLFPPKPKDTLMISRTPEVTCVVVDVSHEDPEVKFNWYVDGVEVHNAKTKPREEQYNSTYRVVSVLTVLHQDWLNGKEYKCKVSNKALPAPIEKTISKAKGQPREPQVYTLPPSRDELTKNQVSLTCLVKGFYPSDIAVEWESNGQPENNYKTTPPVLDSDGSFFLYSKLTVDKSRWQQGNVFSCSVMHEALHNHYTQKSLSLSPGKGSSSSGSSSSSLSCRKEQGKFYDHLLRDCISCASICGQHPKQCAYFCEN

SEQ ID NO: 30 - protein, 505 aa, synthetic construct
QVQLVQSGAEVKKPGASVKVSCKASGYTFTDFAVHWVRQAPGQRLEWMGLIGTSSGSTNYNQKFQGRATMTVDKSANTAYMELSSLRSEDTAVYYCARNGYYVGYYALDYWGQGTTVTVSSASTKGPSVFPLAPSSKSTSGGTAALGCLVKDYFPEPVTVSWNSGALTSGVHTFPAVLQSSGLYSLSSVVTVPSSSLGTQTYICNVNHKPSNTKVDKKVEPKSCDKTHTCPPCPAPELLGGPSVFLFPPKPKDTLMISRTPEVTCVVVDVSHEDPEVKFNWYVDGVEVHNAKTKPREEQYNSTYRVVSVLTVLHQDWLNGKEYKCKVSNKALPAPIEKTISKAKGQPREPQVYTLPPSRDELTKNQVSLTCLVKGFYPSDIAVEWESNGQPENNYKTTPPVLDSDGSFFLYSKLTVDKSRWQQGNVFSCSVMHEALHNHYTQKSLSLSPGKGSSSSGSSSSGSSSSSLSCRKEQGKFYDHLLRDCISCASICGQHPKQCAYFCEN

SEQ ID NO: 31 - protein, 509 aa, synthetic construct
QVQLVQSGAEVKKPGASVKVSCKASGYTFTDFAVHWVRQAPGQRLEWMGLIGTSSGSTNYNQKFQGRATMTVDKSANTAYMELSSLRSEDTAVYYCARNGYYVGYYALDYWGQGTTVTVSSASTKGPSVFPLAPSSKSTSGGTAALGCLVKDYFPEPVTVSWNSGALTSGVHTFPAVLQSSGLYSLSSVVTVPSSSLGTQTYICNVNHKPSNTKVDKKVEPKSCDKTHTCPPCPAPELLGGPSVFLFPPKPKDTLMISRTPEVTCVVVDVSHEDPEVKFNWYVDGVEVHNAKTKPREEQYNSTYRVVSVLTVLHQDWLNGKEYKCKVSNKALPAPIEKTISKAKGQPREPQVYTLPPSRDELTKNQVSLTCLVKGFYPSDIAVEWESNGQPENNYKTTPPVLDSDGSFFLYSKLTVDKSRWQQGNVFSCSVMHEALHNHYTQKSLSLSPGKGGGGSGGGGSGGGGSSLSCRKEQGKFYDHLLRDCISCASICGQHPKQCAYFCENSSSS

SEQ ID NO: 32 - protein, 513 aa, synthetic construct
QVQLVQSGAEVKKPGASVKVSCKASGYTFTDFAVHWVRQAPGQRLEWMGLIGTSSGSTNYNQKFQGRATMTVDKSANTAYMELSSLRSEDTAVYYCARNGYYVGYYALDYWGQGTTVTVSSASTKGPSVFPLAPSSKSTSGGTAALGCLVKDYFPEPVTVSWNSGALTSGVHTFPAVLQSSGLYSLSSVVTVPSSSLGTQTYICNVNHKPSNTKVDKKVEPKSCDKTHTCPPCPAPELLGGPSVFLFPPKPKDTLMISRTPEVTCVVVDVSHEDPEVKFNWYVDGVEVHNAKTKPREEQYNSTYRVVSVLTVLHQDWLNGKEYKCKVSNKALPAPIEKTISKAKGQPREPQVYTLPPSRDELTKNQVSLTCLVKGFYPSDIAVEWESNGQPENNYKTTPPVLDSDGSFFLYSKLTVDKSRWQQGNVFSCSVMHEALHNHYTQKSLSLSPGKGGGGSGGGGSGGGGSSLSCRKEQGKFYDHLLRDCISCASICGQHPKQCAYFCENSSSSSSSS

SEQ ID NO: 33 - protein, 5 aa, synthetic construct
SSTMS

SEQ ID NO: 34 - protein, 17 aa, synthetic construct
TTGGGGSYTYNPDSVKG

SEQ ID NO: 35 - protein, 12 aa, synthetic construct
DRYDGYYFSMDF

SEQ ID NO: 36 - protein, 15 aa, synthetic construct
KASQSVDYDGDSYMN

SEQ ID NO: 37 - protein, 7 aa, synthetic construct
AASNLES

SEQ ID NO: 38 - protein, 9 aa, synthetic construct
QQSNEDPRT

SEQ ID NO: 39 - protein, 6 aa, synthetic construct
DFAVHW

SEQ ID NO: 40 - protein, 17 aa, synthetic construct
LIGTSSGSTNYNQKFKD

SEQ ID NO: 41 - protein, 12 aa, synthetic construct
NGYYVGYYALDY

SEQ ID NO: 42 - protein, 10 aa, synthetic construct
SASSSVSYMY

SEQ ID NO: 43 - protein, 7 aa, synthetic construct
STSNLAS

SEQ ID NO: 44 - protein, 9 aa, synthetic construct
QQRRNYPHT

SEQ ID NO: 45 - protein, 175 aa, synthetic construct
HHHHHHNFMYSKTVKRLSKLREYQQYHPSLTCVMEGKDIEDWSCCPTPWTSFQSSCYFISTGMQSWTKSQKNCSVMGADLVVINTREEQDFIIQNLKRNSSYFLGLSDPGGRRHWQWVDQTPYNENVTFWHSGEPNNLDERCAIINFRSSEEWGWNDIHCHVPQKSICKMKKIYI

SEQ ID NO: 46 - protein, 174 aa, synthetic construct
HHHHHHNFMYSKTVKRLSKLQEYQQYYPSLTCVMEGKDMEDWSCCPTPWTSFQSSCYFISTVMQSWTKSQNNCSVMGAGLVVINTKEEQDFITQNLKINSAYFLGLSDPKGWRHWQWVDQTPYNKNVTFWHSGEPNSPDERCAIINFRSEEWGWNDVHCHVPQKSICKMKKIYI

SEQ ID NO: 47 - protein, 212 aa, synthetic construct
MVPEEEPQDREKGVWWFQLKVWSVAVVSILLLCVCFTVSSVASHNFMYSKTVKRLSKLQEYQQYYPSLTCVMEGKDMEDWSCCPTPWTSFQSSCYFISTVMQSWTKSQNNCSVMGADLVVINTKEEQDFITQNLKINSAYFLGLSDPKGWRHWQWVDQTPYNKNVTFWHSGEPNSPDERCAIINFRSEEWGWNDVHCHVPQKSICKMKKIYI

SEQ ID NO: 48 - protein, 10 aa, synthetic construct
RASSSVSYMY

SEQ ID NO: 49 - protein, 17 aa, synthetic construct
LIGTSSGSTNYNQKFQG

SEQ ID NO: 50 - protein, 499 aa, synthetic construct
QVQLVQSGAEVKKPGASVKVSCKASGYTFTDFAVHWVRQAPGQRLEWMGLIGTSSGSTNYNQKFQGRATMTVDKSANTAYMELSSLRSEDTAVYYCARNGYYVGYYALDYWGQGTTVTVSSASTKGPSVFPLAPSSKSTSGGTAALGCLVKDYFPEPVTVSWNSGALTSGVHTFPAVLQSSGLYSLSSVVTVPSSSLGTQTYICNVNHKPSNTKVDKKVEPKSCDKTHTCPPCPAPELLGGPSVFLFPPKPKDTLMISRTPEVTCVVVDVSHEDPEVKFNWYVDGVEVHNAKTKPREEQYNSTYRVVSVLTVLHQDWLNGKEYKCKVSNKALPAPIEKTISKAKGQPREPQVYTLPPSRDELTKNQVSLTCLVKGFYPSDIAVEWESNGQPENNYKTTPPVLDSDGSFFLYSKLTVDKSRWQQGNVFSCSVMHEALHNHYTQKSLSLSGGGGSGGGGSGGGGSCRKEQGKFYDHLLRDCISCASICGQHPKQCAYFCEN

SEQ ID NO: 51 - protein, 503 aa, synthetic construct
SLSCRKEQGKFYDHLLRDCISCASICGQHPKQCAYFCGGGGSGGGGSGGGGSQVQLVQSGAEVKKPGASVKVSCKASGYTFTDFAVHWVRQAPGQRLEWMGLIGTSSGSTNYNQKFQGRATMTVDKSANTAYMELSSLRSEDTAVYYCARNGYYVGYYALDYWGQGTTVTVSSASTKGPSVFPLAPSSKSTSGGTAALGCLVKDYFPEPVTVSWNSGALTSGVHTFPAVLQSSGLYSLSSVVTVPSSSLGTQTYICNVNHKPSNTKVDKKVEPKSCDKTHTCPPCPAPELLGGPSVFLFPPKPKDTLMISRTPEVTCVVVDVSHEDPEVKFNWYVDGVEVHNAKTKPREEQYNSTYRVVSVLTVLHQDWLNGKEYKCKVSNKALPAPIEKTISKAKGQPREPQVYTLPPSRDELTKNQVSLTCLVKGFYPSDIAVEWESNGQPENNYKTTPPVLDSDGSFFLYSKLTVDKSRWQQGNVFSCSVMHEALHNHYTQKSLSLSPGK

SEQ ID NO: 52 - protein, 213 aa, synthetic construct; identical to SEQ ID NO: 18

SEQ ID NO: 53 - protein, 505 aa, synthetic construct
SLSCRKEQGKFYDHLLRDCISCASICGQHPKQCAYFCENGGGGSGGGGSGGGGSQVQLVQSGAEVKKPGASVKVSCKASGYTFTDFAVHWVRQAPGQRLEWMGLIGTSSGSTNYNQKFQGRATMTVDKSANTAYMELSSLRSEDTAVYYCARNGYYVGYYALDYWGQGTTVTVSSASTKGPSVFPLAPSSKSTSGGTAALGCLVKDYFPEPVTVSWNSGALTSGVHTFPAVLQSSGLYSLSSVVTVPSSSLGTQTYICNVNHKPSNTKVDKKVEPKSCDKTHTCPPCPAPELLGGPSVFLFPPKPKDTLYITREPEVTCVVVDVSHEDPEVKFNWYVDGVEVHNAKTKPREEQYNSTYRVVSVLTVLHQDWLNGKEYKCKVSNKALPAPIEKTISKAKGQPREPQVYTLPPSRDELTKNQVSLTCLVKGFYPSDIAVEWESNGQPENNYKTTPPVLDSDGSFFLYSKLTVDKSRWQQGNVFSCSVMHEALHNHYTQKSLSLSPGK

SEQ ID NO: 54 - protein, 330 aa, synthetic construct
ASTKGPSVFPLAPSSKSTSGGTAALGCLVKDYFPEPVTVSWNSGALTSGVHTFPAVLQSSGLYSLSSVVTVPSSSLGTQTYICNVNHKPSNTKVDKKVEPKSCDKTHTCPPCPAPELLGGPSVFLFPPKPKDTLYITREPEVTCVVVDVSHEDPEVKFNWYVDGVEVHNAKTKPREEQYNSTYRVVSVLTVLHQDWLNGKEYKCKVSNKALPAPIEKTISKAKGQPREPQVYTLPPSRDELTKNQVSLTCLVKGFYPSDIAVEWESNGQPENNYKTTPPVLDSDGSFFLYSKLTVDKSRWQQGNVFSCSVMHEALHNHYTQKSLSLSPGK